European Patent Specification EP 4 158 340 B1, published March 19, 2025. Title: Analyte Detection Method. Applicant: Imperial College Innovations Limited. The sequence listing filed with the application follows.

SEQUENCE LISTING (10 sequences)

SEQ ID NO: 1 - DNA, 25 bp, artificial sequence
  artifical sequence
tttttttttttaggttcccgataac

SEQ ID NO: 2 - DNA, 25 bp, artificial sequence
  artifical sequence
ttttttttttgttatcgggaaccta

SEQ ID NO: 3 - DNA, 107 bp, artificial sequence
  artifical sequence
ttttttttttgttcagtaactaattaacgttgaaatgtccgtaagaacaggaaatcaccaatagactcgacttggatacgcagtgaatatgtctatgcgtatcaatg

SEQ ID NO: 4 - DNA, 35 bp, artificial sequence
  artifical sequence
ttttttttttcattgatacgcatagacatattcac

SEQ ID NO: 5 - DNA, 130 bp, artificial sequence
  artifical sequence
ttttttttttgtccagtggctaattaacgttgaaatgtccgtaagaacaggacatcaccaatagcctcgacttggatacgcagtgcatacgtctacgcgtaggttggtgtggttggatcgtccgtcaatg

SEQ ID NO: 6 - DNA, 26 bp, artificial sequence
  artifical sequence
ttttttttttcattgatacgcgtaga

SEQ ID NO: 7 - RNA, 22 nt, artificial sequence
  artifical sequence
uaacacugucugguaaagaugg

SEQ ID NO: 8 - DNA, 32 bp, artificial sequence
  artifical sequence
tttttccatctttaccagacagtgttattttt

SEQ ID NO: 9 - RNA, 22 nt, artificial sequence
  artifical sequence
uaacacugucugguaacgaugu

SEQ ID NO: 10 - DNA, 15 bp, artificial sequence
  artifical sequence
ggttggtgtggttgg